European Patent Specification EP 4 078 180 B1, published July 29, 2026. Title: A library of prefabricated microparticles and precursors thereof. Applicant: Blink AG. The sequence listing filed with the application follows.

SEQUENCE LISTING (8 sequences)

SEQ ID NO: 1 - DNA, 24 bp, Artificial Sequence
  "desthiobiotin-labeled rpoB sense primer "
  desthiobiotin-labeled rpoB sense primer
atcaacatccggccggtggtcgcc

SEQ ID NO: 2 - DNA, 21 bp, Artificial Sequence
  "desthiobiotin-labeled rpoB antisense primer "
  desthiobiotin-labeled rpoB antisense primer
tcacgtgacagaccgccgggc

SEQ ID NO: 3 - DNA, 22 bp, Artificial Sequence
  "desthiobiotin-labeled IS6110 sense primer "
  desthiobiotin-labeled IS6110 sense primer
cgccgcttcggaccaccagcac

SEQ ID NO: 4 - DNA, 25 bp, Artificial Sequence
  "desthiobiotin-labeled IS6110 antisense primer "
  desthiobiotin-labeled IS6110 antisense primer
gtgacaaaggccacgtaggcgaacc

SEQ ID NO: 5 - DNA, 25 bp, Artificial Sequence
  "desthiobiotin-labeled IS1081 sense primer "
  desthiobiotin-labeled IS1081 sense primer
gcgcggcaagatcatcaatgtggag

SEQ ID NO: 6 - DNA, 21 bp, Artificial Sequence
  "desthiobiotin-labeled IS1081 antisense primer "
  desthiobiotin-labeled IS1081 antisense primer
gccaccgcggggagtttgtcg

SEQ ID NO: 7 - DNA, 25 bp, Artificial Sequence
  "desthiobiotin-labeled internal control (Bac. globigii) sense primer"
  desthiobiotin-labeled internal control (Bac. globigii) sense primer
gcgcggcaagatcatcaatgtggag

SEQ ID NO: 8 - DNA, 21 bp, Artificial Sequence
  "desthiobiotin-labeled internal control (Bac. globigii) antisense primer "
  desthiobiotin-labeled internal control (Bac. globigii) antisense primer
gccaccgcggggagtttgtcg